European Patent Specification EP 3 592 771 B1, published September 30, 2026. Title: Monoclonal Antibody against Both IL-17A and IL-17F and Use of the Same. Applicant: X-KANG United Biopharmaceutical Science & Technology Co. Ltd. The sequence listing filed with the application follows.

SEQUENCE LISTING (11 sequences)

SEQ ID NO: 1 - protein, 5 aa, Artificial sequence
  CDR1H amino acid sequence
DYNLN

SEQ ID NO: 2 - protein, 17 aa, Artificial sequence
  CDR2H amino acid sequence
VIHPDYGTTSYNQKFKD

SEQ ID NO: 3 - protein, 9 aa, Artificial sequence
  CDR3H amino acid sequence
YDYGDAMDY

SEQ ID NO: 4 - protein, 16 aa, Artificial sequence
  CDR1L amino acid sequence
RSSQSLVHSNGNTYLH

SEQ ID NO: 5 - protein, 7 aa, Artificial sequence
  CDR2L amino acid sequence
KVSNRFS

SEQ ID NO: 6 - protein, 9 aa, Artificial sequence
  CDR3L amino acid sequence
SQSTHVPLT

SEQ ID NO: 7 - protein, 118 aa, Artificial sequence
  Variable heavy chain domain (VH1-1) amino acid sequence
QFQLVQSGAEVKKPGASVKVSCKASGYTFTDYNLNWVRQAPGKGLEWMGVIHPDYGTTSYNQKFKDRVTMTVDTSTSTVYMELSSLRSEDTAVYYCVRYDYGDAMDYWGQGTLVTVSS

SEQ ID NO: 8 - protein, 112 aa, Artificial sequence
  Variable light chain domain (VL5) amino acid sequence
DIVMTQSPLSLSVTPGQPASISCRSSQSLVHSNGNTYLHWYLQKPGQPPQLLIYKVSNRFSGVPDRFSGSGSGTDFTLKISRVEAEDVGVYYCSQSTHVPLTFGQGTKLEIK

SEQ ID NO: 9 - protein, 112 aa, Artificial sequence
  Variable light chain domain (VL2-1) amino acid sequence
DIVMTQTPLSSSVTLGQPASISCRSSQSLVHSNGNTYLHWLQQRPGQPPRLLIYKVSNRFSGVPDRFSGSGAGTDFTLKISRVEAEDVGVYYCSQSTHVPLTFGQGTKLEIK

SEQ ID NO: 10 - protein, 448 aa, Artificial sequence
  Heavy chain amino acid sequence comprising VH1-1
QFQLVQSGAEVKKPGASVKVSCKASGYTFTDYNLNWVRQAPGKGLEWMGVIHPDYGTTSYNQKFKDRVTMTVDTSTSTVYMELSSLRSEDTAVYYCVRYDYGDAMDYWGQGTLVTVSSASTKGPSVFPLAPSSKSTSGGTAALGCLVKDYFPEPVTVSWNSGALTSGVHTFPAVLQSSGLYSLSSVVTVPSSSLGTQTYICNVNHKPSNTKVDKKVEPKSCDKTHTCPPCPAPELLGGPSVFLFPPKPKDTLMISRTPEVTCVVVDVSHEDPEVKFNWYVDGVEVHNAKTKPREEQYNSTYRVVSVLTVLHQDWLNGKEYKCKVSNKALPAPIEKTISKAKGQPREPQVYTLPPSRDELTKNQVSLTCLVKGFYPSDIAVEWESNGQPENNYKTTPPVLDSDGSFFLYSKLTVDKSRWQQGNVFSCSVMHEALHNHYTQKSLSLSPGK

SEQ ID NO: 11 - protein, 219 aa, Artificial sequence
  Light chain amino acid sequence comprising VL5
DIVMTQSPLSLSVTPGQPASISCRSSQSLVHSNGNTYLHWYLQKPGQPPQLLIYKVSNRFSGVPDRFSGSGSGTDFTLKISRVEAEDVGVYYCSQSTHVPLTFGQGTKLEIKRTVAAPSVFIFPPSDEQLKSGTASVVCLLNNFYPREAKVQWKVDNALQSGNSQESVTEQDSKDSTYSLSSTLTLSKADYEKHKVYACEVTHQGLSSPVTKSFNRGEC